European Patent Application EP 4 368 253 A1, published May 15, 2024. Title: Metal-binding polypeptide. Applicant: Eberhard Karls Universität Tübingen - Medizinische Fakultät. The sequence listing filed with the application follows.

SEQUENCE LISTING (9 sequences)

SEQ ID NO: 1 - protein, 110 aa, Methylosinus trichosporium
MGAKYKALLDSSSHCVAVGEDCLRHCFEMLAMNDASMGACTKATYDLVAACGALAKLAGTNSAFTPAFAKVVADVCAACKKECDKFPSIAECKACGEACQACAEECHKVA

SEQ ID NO: 2 - protein, 111 aa, synthetic construct
XXGAXYXALLXSSXXCVXVGEXXLXHXXEMLXXNDXSMGAXTKAXXDLVXACXXLAKLAGTXSAXTPXXAXXVAXVCXXCXKEXDKXPSXXEXKXXXEACXXCAEECXKVA

SEQ ID NO: 3 - protein, 110 aa, synthetic construct
MGAKYKALLESSRRCVRVGERCLRHCREMLRRNDASMGACTKATYDLVKACAELAKLAGTNSARTPKKAKQVARVCEKCKKECDKFPSIAECKACAEACKKCAEECRKVA

SEQ ID NO: 4 - protein, 110 aa, synthetic construct
MGAKYKALLRSSRRCVKVGEECLRHCREMLKRNDASMGACTKATYDLVKACARLAKLAGTNSARTPRRAKRVARVCERCKKECDKFPSIAECKACAEACQRCAEECKKVA

SEQ ID NO: 5 - protein, 111 aa, synthetic construct
MHGAKYKALLESSRRCVRVGERCLRHAREMLRRNDASMGALTKATYDLVKACAELAKLAGTNSARTPKKAKQVARVCEKCKKECDKWPSMAEAKACAEACKKCAEECRKVA

SEQ ID NO: 6 - protein, 111 aa, synthetic construct
MHGAKYKALLESSRRCVRVGERALRHAREMLRRNDASMGAATKAFYDLVKACAELAKLAGTNSARTPKKAKQVARVCEKCKKEADKWPSYAEAKAAAEACKKCAEECRKVA

SEQ ID NO: 7 - protein, 111 aa, synthetic construct
MHGAKYKALLESSRRCVRVGERWLRHAREMLRRNDASMGAATKAAYDLVKACAELAKLAGTNSARTPKKAKQVARVCEKCKKEADKWPSMAEAKAAAEACKKCAEECRKVA

SEQ ID NO: 8 - protein, 111 aa, synthetic construct
MHGAHYAALLESSERCVEVGERCLEHCQEMLEKNDESMGACTKATEDLVKACEELAKLAGTESAQTPELAAEVARVCEQCQKECDKFPSIEECKECAEACQECAEECEKVA

SEQ ID NO: 9 - protein, 111 aa, synthetic construct
MHGAHYEALLESSERCVEVGERCLEHCQEMLEKNDESMGACTKATEDLVKACEELAKLAGTESAQTPELAAEVARVCRQCAKECDKFPSIEECKECAEACEECAEECRKVA